European Patent Application EP 4 190 352 A1, published June 7, 2023. Title: NOVEL BISPECIFIC ANTI-CD3/CD20 POLYPEPTIDE COMPLEX FORMULATION. Applicant: Chia Tai Tianqing Pharmaceutical Group Co., Ltd. The sequence listing filed with the application follows.

SEQUENCE LISTING (62 sequences)

SEQ ID NO: 1 - protein, 10 aa, Artificial Sequence
  CDR1
GYSFTTYYIH

SEQ ID NO: 2 - protein, 17 aa, Artificial Sequence
  CDR2
WIFPGNDNIKYSEKFKG

SEQ ID NO: 3 - protein, 10 aa, Artificial Sequence
  CDR3
DSVSIYYFDY

SEQ ID NO: 4 - protein, 17 aa, Artificial Sequence
  CDR1
KSSQSLLNSRTRKNYLA

SEQ ID NO: 5 - protein, 7 aa, Artificial Sequence
  CDR2
WASTRKS

SEQ ID NO: 6 - protein, 8 aa, Artificial Sequence
  CDR3
TQSFILRT

SEQ ID NO: 7 - protein, 10 aa, Artificial Sequence
  CDR1
GFTFNDYAMH

SEQ ID NO: 8 - protein, 17 aa, Artificial Sequence
  CDR2
TISWNSGSIGYADSVKG

SEQ ID NO: 9 - protein, 13 aa, Artificial Sequence
  CDR3
DIQYGNYYYGMDV

SEQ ID NO: 10 - protein, 11 aa, Artificial Sequence
  CDR1
RASQSVSSYLA

SEQ ID NO: 11 - protein, 7 aa, Artificial Sequence
  CDR2
DASNRAT

SEQ ID NO: 12 - protein, 9 aa, Artificial Sequence
  CDR3
QQRSNWPIT

SEQ ID NO: 13 - protein, 10 aa, Artificial Sequence
  CDR1
GFAFTDYYIH

SEQ ID NO: 14 - protein, 17 aa, Artificial Sequence
  CDR2
WISPGNVNTKYNENFKG

SEQ ID NO: 15 - protein, 10 aa, Artificial Sequence
  CDR3
DGYSLYYFDY

SEQ ID NO: 16 - protein, 17 aa, Artificial Sequence
  CDR1
KSSQSLLNSRTRKNYLA

SEQ ID NO: 17 - protein, 7 aa, Artificial Sequence
  CDR2
WASTRQS

SEQ ID NO: 18 - protein, 8 aa, Artificial Sequence
  CDR3
TQSHTLRT

SEQ ID NO: 19 - protein, 10 aa, Artificial Sequence
  CDR1
GYTFTSYNMH

SEQ ID NO: 20 - protein, 17 aa, Artificial Sequence
  CDR2
AIYPGNGDTSYNQKFKG

SEQ ID NO: 21 - protein, 12 aa, Artificial Sequence
  CDR3
STYYGGDWYFNV

SEQ ID NO: 22 - protein, 10 aa, Artificial Sequence
  CDR1
RASSSVSYIH

SEQ ID NO: 23 - protein, 7 aa, Artificial Sequence
  CDR2
ATSNLAS

SEQ ID NO: 24 - protein, 9 aa, Artificial Sequence
  CDR3
QQWTSNPPT

SEQ ID NO: 25 - protein, 119 aa, Artificial Sequence
  VH
QVQLVQSGAEVKKPGSSVKVSCKASGYSFTTYYIHWVRQAPGQGLEWMGWIFPGNDNIKYSEKFKGRVTITADKSTSTAYMELSSLRSEDTAVYYCAIDSVSIYYFDYWGQGTLVTVSS

SEQ ID NO: 26 - protein, 112 aa, Artificial Sequence
  Vκ
DIVMTQSPDSLAVSLGERATINCKSSQSLLNSRTRKNYLAWYQQKPGQPPKLLIYWASTRKSGVPDRFSGSGSGTDFTLTISSLQAEDVAVYYCTQSFILRTFGGGTKVEIK

SEQ ID NO: 27 - protein, 119 aa, Artificial Sequence
  VH
QVQLVQSGAEVKKPGSSVKVSCKASGFAFTDYYIHWVRQAPGQGLEWMGWISPGNVNTKYNENFKGRVTITADKSTSTAYMELSSLRSEDTAVYYCARDGYSLYYFDYWGQGTLVTVSS

SEQ ID NO: 28 - protein, 112 aa, Artificial Sequence
  Vκ
DIVMTQSPDSLAVSLGERATINCKSSQSLLNSRTRKNYLAWYQQKPGQPPKLLIYWASTRQSGVPDRFSGSGSGTDFTLTISSLQAEDVAVYYCTQSHTLRTFGGGTKVEIK

SEQ ID NO: 29 - protein, 122 aa, Artificial Sequence
  VH
EVQLVESGGGLVQPGRSLRLSCAASGFTFNDYAMHWVRQAPGKGLEWVSTISWNSGSIGYADSVKGRFTISRDNAKKSLYLQMNSLRAEDTALYYCAKDIQYGNYYYGMDVWGQGTTVTVSS

SEQ ID NO: 30 - protein, 107 aa, Artificial Sequence
  Vκ
EIVLTQSPATLSLSPGERATLSCRASQSVSSYLAWYQQKPGQAPRLLIYDASNRATGIPARFSGSGSGTDFTLTISSLEPEDFAVYYCQQRSNWPITFGQGTRLEIK

SEQ ID NO: 31 - protein, 121 aa, Artificial Sequence [sequence omitted]

SEQ ID NO: 32 - protein, 106 aa, Artificial Sequence [sequence omitted]

SEQ ID NO: 33 - protein, 445 aa, Artificial Sequence
  H1
QVQLVQSGAEVKKPGSSVKVSCKASGYSFTTYYIHWVRQAPGQGLEWMGWIFPGNDNIKYSEKFKGRVTITADKSTSTAYMELSSLRSEDTAVYYCAIDSVSIYYFDYWGQGTLVTVSSASTKGPSVFPLAPCSRSTSESTAALGCLVKDYFPEPVTVSWNSGALTSGVHTFPAVLQSSGLYSLSSVVTVPSSSLGTKTYTCNVDHKPSNTKVDKRVESKYGPPCPPCPAPEFLGGPSVFLFPPKPKDTLMISRTPEVTCVVVDVSQEDPEVQFNWYVDGVEVHNAKTKPREEQFNSTYRVVSVLTVLHQDWLNGKEYKCKVSNKGLPSSIEKTISKAKGQPREPQVYTLPPCQEEMTKNQVSLWCLVKGFYPSDIAVEWESNGQPENNYKTTPPVLDSDGSFFLYSRLTVDKSRWQEGNVFSCSVMHEALHNHYTQKSLSLSLG

SEQ ID NO: 34 - protein, 474 aa, Artificial Sequence
  H2
EVQLVESGGGLVQPGRSLRLSCAASGFTFNDYAMHWVRQAPGKGLEWVSTISWNSGSIGYADSVKGRFTISRDNAKKSLYLQMNSLRAEDTALYYCAKDIQYGNYYYGMDVWGQGTTVTVLEDLKNVFPPEVAVFEPSEAEISHTQKATLVCLATGFYPDHVELSWWVNGKEVHSGVCTDPQPLKEQPALQDSRYALSSRLRVSATFWQNPRNHFRCQVQFYGLSENDEWTQDRAKPVTQIVSAEAWGRYGPPCPPCPAPEFLGGPSVFLFPPKPKDTLMISRTPEVTCVVVDVSQEDPEVQFNWYVDGVEVHNAKTKPREEQFNSTYRVVSVLTVLHQDWLNGKEYKCKVSNKGLPSSIEKTISKAKGQPREPQVCTLPPSQEEMTKNQVSLSCAVKGFYPSDIAVEWESNGQPENNYKTTPPVLDSDGSFFLVSRLTVDKSRWQEGNVFSCSVMHEALHNHYTQKSLSLSLG

SEQ ID NO: 35 - protein, 219 aa, Artificial Sequence
  L1
DIVMTQSPDSLAVSLGERATINCKSSQSLLNSRTRKNYLAWYQQKPGQPPKLLIYWASTRKSGVPDRFSGSGSGTDFTLTISSLQAEDVAVYYCTQSFILRTFGGGTKVEIKRTVAAPSVFIFPPSDEQLKSGTASVVCLLNNFYPREAKVQWKVDNALQSGNSQESVTEQDSKDSTYSLSSTLTLSKADYEKHKVYACEVTHQGLSSPVTKSFNRGEC

SEQ ID NO: 36 - protein, 202 aa, Artificial Sequence
  L2
EIVLTQSPATLSLSPGERATLSCRASQSVSSYLAWYQQKPGQAPRLLIYDASNRATGIPARFSGSGSGTDFTLTISSLEPEDFAVYYCQQRSNWPITFGQGTRLEIKPDIQNPDPAVYQLRDSKSSDKSVCLFTDFDSQTQVSQSKDSDVYITDKCVLDMRSMDFKSNSAVAWSQKSDFACANAFQNSIIPEDTFFPSPESS

SEQ ID NO: 37 - protein, 471 aa, Artificial Sequence
  H1
QVQLVQSGAEVKKPGSSVKVSCKASGFAFTDYYIHWVRQAPGQGLEWMGWISPGNVNTKYNENFKGRVTITADKSTSTAYMELSSLRSEDTAVYYCARDGYSLYYFDYWGQGTLVTVLEDLKNVFPPEVAVFEPSEAEISHTQKATLVCLATGFYPDHVELSWWVNGKEVHSGVCTDPQPLKEQPALQDSRYALSSRLRVSATFWQNPRNHFRCQVQFYGLSENDEWTQDRAKPVTQIVSAEAWGRYGPPCPPCPAPEFLGGPSVFLFPPKPKDTLMISRTPEVTCVVVDVSQEDPEVQFNWYVDGVEVHNAKTKPREEQFNSTYRVVSVLTVLHQDWLNGKEYKCKVSNKGLPSSIEKTISKAKGQPREPQVYTLPPCQEEMTKNQVSLWCLVKGFYPSDIAVEWESNGQPENNYKTTPPVLDSDGSFFLYSRLTVDKSRWQEGNVFSCSVMHEALHNHYTQKSLSLSLG

SEQ ID NO: 38 - protein, 676 aa, Artificial Sequence
  H2
QVQLQQPGAELVKPGASVKMSCKASGYTFTSYNMHWVKQTPGRGLEWIGAIYPGNGDTSYNQKFKGKATLTADKSSSTAYMQLSSLTSEDSAVYYCARSTYYGGDWYFNVWGAGTTVTVSAASTKGPSVFPLAPCSRSTSESTAALGCLVKDYFPEPVTVSWNSGALTSGVHTFPAVLQSSGLYSLSSVVTVPSSSLGTKTYTCNVDHKPSNTKVDKRVGGGGSGGGGSQVQLQQPGAELVKPGASVKMSCKASGYTFTSYNMHWVKQTPGRGLEWIGAIYPGNGDTSYNQKFKGKATLTADKSSSTAYMQLSSLTSEDSAVYYCARSTYYGGDWYFNVWGAGTTVTVSAASTKGPSVFPLAPCSRSTSESTAALGCLVKDYFPEPVTVSWNSGALTSGVHTFPAVLQSSGLYSLSSVVTVPSSSLGTKTYTCNVDHKPSNTKVDKRVESKYGPPCPPCPAPEFLGGPSVFLFPPKPKDTLMISRTPEVTCVVVDVSQEDPEVQFNWYVDGVEVHNAKTKPREEQFNSTYRVVSVLTVLHQDWLNGKEYKCKVSNKGLPSSIEKTISKAKGQPREPQVCTLPPSQEEMTKNQVSLSCAVKGFYPSDIAVEWESNGQPENNYKTTPPVLDSDGSFFLVSRLTVDKSRWQEGNVFSCSVMHEALHNHYTQKSLSLSLG

SEQ ID NO: 39 - protein, 207 aa, Artificial Sequence
  L1
DIVMTQSPDSLAVSLGERATINCKSSQSLLNSRTRKNYLAWYQQKPGQPPKLLIYWASTRQSGVPDRFSGSGSGTDFTLTISSLQAEDVAVYYCTQSHTLRTFGGGTKVEIKPDIQNPDPAVYQLRDSKSSDKSVCLFTDFDSQTQVSQSKDSDVYITDKCVLDMRSMDFKSNSAVAWSQKSDFACANAFQNSIIPEDTFFPSPESS

SEQ ID NO: 40 - protein, 213 aa, Artificial Sequence
  L2
QIVLSQSPAILSASPGEKVTMTCRASSSVSYIHWFQQKPGSSPKPWIYATSNLASGVPVRFSGSGSGTSYSLTISRVEAEDAATYYCQQWTSNPPTFGGGTKLEIKRTVAAPSVFIFPPSDEQLKSGTASVVCLLNNFYPREAKVQWKVDNALQSGNSQESVTEQDSKDSTYSLSSTLTLSKADYEKHKVYACEVTHQGLSSPVTKSFNRGEC

SEQ ID NO: 41 - protein, 700 aa, Artificial Sequence
  H1
QVQLQQPGAELVKPGASVKMSCKASGYTFTSYNMHWVKQTPGRGLEWIGAIYPGNGDTSYNQKFKGKATLTADKSSSTAYMQLSSLTSEDSAVYYCARSTYYGGDWYFNVWGAGTTVTVSAASTKGPSVFPLAPCSRSTSESTAALGCLVKDYFPEPVTVSWNSGALTSGVHTFPAVLQSSGLYSLSSVVTVPSSSLGTKTYTCNVDHKPSNTKVDKRVGGGGSGGGGSQVQLVQSGAEVKKPGSSVKVSCKASGFAFTDYYIHWVRQAPGQGLEWMGWISPGNVNTKYNENFKGRVTITADKSTSTAYMELSSLRSEDTAVYYCARDGYSLYYFDYWGQGTLVTVLEDLKNVFPPEVAVFEPSEAEISHTQKATLVCLATGFYPDHVELSWWVNGKEVHSGVCTDPQPLKEQPALQDSRYALSSRLRVSATFWQNPRNHFRCQVQFYGLSENDEWTQDRAKPVTQIVSAEAWGRYGPPCPPCPAPEFLGGPSVFLFPPKPKDTLMISRTPEVTCVVVDVSQEDPEVQFNWYVDGVEVHNAKTKPREEQFNSTYRVVSVLTVLHQDWLNGKEYKCKVSNKGLPSSIEKTISKAKGQPREPQVYTLPPCQEEMTKNQVSLWCLVKGFYPSDIAVEWESNGQPENNYKTTPPVLDSDGSFFLYSRLTVDKSRWQEGNVFSCSVMHEALHNHYTQKSLSLSLG

SEQ ID NO: 42 - protein, 447 aa, Artificial Sequence
  H2
QVQLQQPGAELVKPGASVKMSCKASGYTFTSYNMHWVKQTPGRGLEWIGAIYPGNGDTSYNQKFKGKATLTADKSSSTAYMQLSSLTSEDSAVYYCARSTYYGGDWYFNVWGAGTTVTVSAASTKGPSVFPLAPCSRSTSESTAALGCLVKDYFPEPVTVSWNSGALTSGVHTFPAVLQSSGLYSLSSVVTVPSSSLGTKTYTCNVDHKPSNTKVDKRVESKYGPPCPPCPAPEFLGGPSVFLFPPKPKDTLMISRTPEVTCVVVDVSQEDPEVQFNWYVDGVEVHNAKTKPREEQFNSTYRVVSVLTVLHQDWLNGKEYKCKVSNKGLPSSIEKTISKAKGQPREPQVCTLPPSQEEMTKNQVSLSCAVKGFYPSDIAVEWESNGQPENNYKTTPPVLDSDGSFFLVSRLTVDKSRWQEGNVFSCSVMHEALHNHYTQKSLSLSLG

SEQ ID NO: 43 - protein, 213 aa, Artificial Sequence; identical to SEQ ID NO: 40
  L1

SEQ ID NO: 44 - protein, 207 aa, Artificial Sequence; identical to SEQ ID NO: 39
  L2

SEQ ID NO: 45 - protein, 701 aa, Artificial Sequence
  H1
EVQLVESGGGLVQPGRSLRLSCAASGFTFNDYAMHWVRQAPGKGLEWVSTISWNSGSIGYADSVKGRFTISRDNAKKSLYLQMNSLRAEDTALYYCAKDIQYGNYYYGMDVWGQGTTVTVSSASTKGPSVFPLAPCSRSTSESTAALGCLVKDYFPEPVTVSWNSGALTSGVHTFPAVLQSSGLYSLSSVVTVPSSSLGTKTYTCNVDHKPSNTKVDKRVGGGGSGGGGSQVQLVQSGAEVKKPGSSVKVSCKASGYSFTTYYIHWVRQAPGQGLEWMGWIFPGNDNIKYSEKFKGRVTITADKSTSTAYMELSSLRSEDTAVYYCAIDSVSIYYFDYWGQGTLVTVLEDLKNVFPPEVAVFEPSEAEISHTQKATLVCLATGFYPDHVELSWWVNGKEVHSGVCTDPQPLKEQPALQDSRYALSSRLRVSATFWQNPRNHFRCQVQFYGLSENDEWTQDRAKPVTQIVSAEAWGRYGPPCPPCPAPEFLGGPSVFLFPPKPKDTLMISRTPEVTCVVVDVSQEDPEVQFNWYVDGVEVHNAKTKPREEQFNSTYRVVSVLTVLHQDWLNGKEYKCKVSNKGLPSSIEKTISKAKGQPREPQVYTLPPCQEEMTKNQVSLWCLVKGFYPSDIAVEWESNGQPENNYKTTPPVLDSDGSFFLYSRLTVDKSRWQEGNVFSCSVMHEALHNHYTQKSLSLSLG

SEQ ID NO: 46 - protein, 448 aa, Artificial Sequence
  H2
EVQLVESGGGLVQPGRSLRLSCAASGFTFNDYAMHWVRQAPGKGLEWVSTISWNSGSIGYADSVKGRFTISRDNAKKSLYLQMNSLRAEDTALYYCAKDIQYGNYYYGMDVWGQGTTVTVSSASTKGPSVFPLAPCSRSTSESTAALGCLVKDYFPEPVTVSWNSGALTSGVHTFPAVLQSSGLYSLSSVVTVPSSSLGTKTYTCNVDHKPSNTKVDKRVESKYGPPCPPCPAPEFLGGPSVFLFPPKPKDTLMISRTPEVTCVVVDVSQEDPEVQFNWYVDGVEVHNAKTKPREEQFNSTYRVVSVLTVLHQDWLNGKEYKCKVSNKGLPSSIEKTISKAKGQPREPQVCTLPPSQEEMTKNQVSLSCAVKGFYPSDIAVEWESNGQPENNYKTTPPVLDSDGSFFLVSRLTVDKSRWQEGNVFSCSVMHEALHNHYTQKSLSLSLG

SEQ ID NO: 47 - protein, 214 aa, Artificial Sequence
  L1
EIVLTQSPATLSLSPGERATLSCRASQSVSSYLAWYQQKPGQAPRLLIYDASNRATGIPARFSGSGSGTDFTLTISSLEPEDFAVYYCQQRSNWPITFGQGTRLEIKRTVAAPSVFIFPPSDEQLKSGTASVVCLLNNFYPREAKVQWKVDNALQSGNSQESVTEQDSKDSTYSLSSTLTLSKADYEKHKVYACEVTHQGLSSPVTKSFNRGEC

SEQ ID NO: 48 - protein, 207 aa, Artificial Sequence
  L2
DIVMTQSPDSLAVSLGERATINCKSSQSLLNSRTRKNYLAWYQQKPGQPPKLLIYWASTRKSGVPDRFSGSGSGTDFTLTISSLQAEDVAVYYCTQSFILRTFGGGTKVEIKPDIQNPDPAVYQLRDSKSSDKSVCLFTDFDSQTQVSQSKDSDVYITDKCVLDMRSMDFKSNSAVAWSQKSDFACANAFQNSIIPEDTFFPSPESS

SEQ ID NO: 49 - protein, 703 aa, Artificial Sequence
  H1
QVQLVQSGAEVKKPGSSVKVSCKASGFAFTDYYIHWVRQAPGQGLEWMGWISPGNVNTKYNENFKGRVTITADKSTSTAYMELSSLRSEDTAVYYCARDGYSLYYFDYWGQGTLVTVLEDLKNVFPPEVAVFEPSEAEISHTQKATLVCLATGFYPDHVELSWWVNGKEVHSGVCTDPQPLKEQPALQDSRYALSSRLRVSATFWQNPRNHFRCQVQFYGLSENDEWTQDRAKPVTQIVSAEAWGRGGGGSGGGGSQVQLQQPGAELVKPGASVKMSCKASGYTFTSYNMHWVKQTPGRGLEWIGAIYPGNGDTSYNQKFKGKATLTADKSSSTAYMQLSSLTSEDSAVYYCARSTYYGGDWYFNVWGAGTTVTVSAASTKGPSVFPLAPCSRSTSESTAALGCLVKDYFPEPVTVSWNSGALTSGVHTFPAVLQSSGLYSLSSVVTVPSSSLGTKTYTCNVDHKPSNTKVDKRVESKYGPPCPPCPAPEFLGGPSVFLFPPKPKDTLMISRTPEVTCVVVDVSQEDPEVQFNWYVDGVEVHNAKTKPREEQFNSTYRVVSVLTVLHQDWLNGKEYKCKVSNKGLPSSIEKTISKAKGQPREPQVYTLPPCQEEMTKNQVSLWCLVKGFYPSDIAVEWESNGQPENNYKTTPPVLDSDGSFFLYSRLTVDKSRWQEGNVFSCSVMHEALHNHYTQKSLSLSLG

SEQ ID NO: 50 - protein, 447 aa, Artificial Sequence; identical to SEQ ID NO: 42
  H2

SEQ ID NO: 51 - protein, 207 aa, Artificial Sequence; identical to SEQ ID NO: 39
  L1

SEQ ID NO: 52 - protein, 213 aa, Artificial Sequence; identical to SEQ ID NO: 40
  L2

SEQ ID NO: 53 - DNA, 357 bp, Artificial Sequence
  VH
caggtgcaactcgtgcagtctggagctgaagtgaagaagcctgggtcttcagtcaaggtcagttgcaaggccagtgggtattccttcactacctactacatccactgggtgcggcaggcaccaggacaggggcttgagtggatgggctggatctttcccggcaacgataatattaagtacagcgagaagttcaaagggagggtcaccattaccgccgacaaatccacttccacagcctacatggagttgagcagcctgagatccgaggatacagccgtgtactactgtgccattgacagcgtgtccatctactactttgactactggggccagggcacactggtcacagtgagcagc

SEQ ID NO: 54 - DNA, 336 bp, Artificial Sequence
  Vκ
gacatcgtcatgacccagtccccagactctttggcagtgtctctcggggaaagagctaccatcaactgcaagagcagccagtcccttctgaacagcaggaccaggaagaattacctcgcctggtaccaacagaagcccggacagcctcctaagctcctgatctactgggcctcaacccggaagagtggagtgcccgatcgctttagcgggagcggctccgggacagatttcacactgacaatttcctccctgcaggccgaggacgtcgccgtgtattactgtactcagagcttcattctgcggacatttggcggcgggactaaagtggagattaag

SEQ ID NO: 55 - DNA, 357 bp, Artificial Sequence
  VH
caggtgcagcttgtgcagtctggggcagaagtgaagaagcctgggtctagtgtcaaggtgtcatgcaaggctagcgggttcgcctttactgactactacatccactgggtgcggcaggctcccggacaagggttggagtggatgggatggatctccccaggcaatgtcaacacaaagtacaacgagaacttcaaaggccgcgtcaccattaccgccgacaagagcacctccacagcctacatggagctgtccagcctcagaagcgaggacactgccgtctactactgtgccagggatgggtactccctgtattactttgattactggggccagggcacactggtgacagtgagctcc

SEQ ID NO: 56 - DNA, 336 bp, Artificial Sequence
  Vκ
gatatcgtgatgacccagagcccagactcccttgctgtctccctcggcgaaagagcaaccatcaactgcaagagctcccaaagcctgctgaactccaggaccaggaagaattacctggcctggtatcagcagaagcccggccagcctcctaagctgctcatctactgggcctccacccggcagtctggggtgcccgatcggtttagtggatctgggagcgggacagacttcacattgacaattagctcactgcaggccgaggacgtggccgtctactactgtactcagagccacactctccgcacattcggcggagggactaaagtggagattaag

SEQ ID NO: 57 - DNA, 366 bp, Artificial Sequence
  VH
gaggtgcaattggtggagagcggaggagggctcgtgcagcctggaagatctcttaggctgagttgcgctgcatctgggttcacattcaacgactacgccatgcactgggtgaggcaggctcccggcaaagggctggaatgggtgtcaactatctcctggaactccggcagcatcggctacgccgatagcgtcaagggccggtttacaatttcccgcgataacgccaagaagtccctgtacctgcagatgaacagcctgcgggccgaggatactgccctctactactgtgccaaggacattcagtacgggaattactattacgggatggacgtctggggccaggggaccaccgtgacagtcagctcc

SEQ ID NO: 58 - DNA, 321 bp, Artificial Sequence
  Vκ
gaaatcgtgctgacccagtccccagcaaccctctccctttctcctggagagagagctaccctcagctgtagggcctcacagtctgtctccagttacctggcttggtaccagcagaaacccgggcaggcccctaggttgctgatctacgacgccagcaatagggccactggcatcccagcccggttttccggaagcggcagcgggacagatttcacactcactattagcagcctggagcccgaggacttcgccgtgtactattgccagcagcggtccaactggcccattacatttggccaagggacacgcctggagattaag

SEQ ID NO: 59 - DNA, 363 bp, Artificial Sequence
  VH
caggtccagctgcagcagcccggagccgaactggtcaaacccggggctagcgtgaaaatgtcttgcaaagcaagtggttacacattcacttcctataacatgcactgggtgaagcagacacctgggcgaggtctggaatggatcggcgccatctacccaggcaacggagacactagctataatcagaagtttaaaggaaaggccaccctgacagctgataagtccagctctaccgcttacatgcagctgagttcactgacaagtgaggactcagcagtgtactattgcgcccgttctacctactatggcggagattggtatttcaatgtgtggggcgccggtaccacagtcaccgtgtccgcc

SEQ ID NO: 60 - DNA, 318 bp, Artificial Sequence
  Vκ
cagattgtcctgagccagagccctgccatcctgtctgctagtcccggcgagaaggtgaccatgacatgcagggcatccagctctgtctcctacatccactggttccagcagaagcccgggagttcacctaaaccatggatctacgctacatccaacctggcaagcggtgtgcctgtcaggttttcaggttccggcagcggaacatcttacagtctgactatttctcgggtggaggccgaagacgccgctacctactattgccagcagtggacctccaatccccctacattcggcggagggactaagctggagatcaaa

SEQ ID NO: 61 - protein, 126 aa, Artificial Sequence
  Engineered Cβ (engineered TCRBeta)
LEDLKNVFPPEVAVFEPSEAEISHTQKATLVCLATGFYPDHVELSWWVNGKEVHSGVCTDPQPLKEQPALQDSRYALSSRLRVSATFWQNPRNHFRCQVQFYGLSENDEWTQDRAKPVTQIVSAEA

SEQ ID NO: 62 - protein, 95 aa, Artificial Sequence
  Engineered Cα (engineered TCRAlpha)
PDIQNPDPAVYQLRDSKSSDKSVCLFTDFDSQTQVSQSKDSDVYITDKCVLDMRSMDFKSNSAVAWSQKSDFACANAFQNSIIPEDTFFPSPESS